European Patent Application EP 4 112 078 A1, published January 4, 2023. Title: The IgM and IgE heavy chain domain 2 as covalently linked homodimerization modules for the generation of fusion proteins with dual specificity. Applicant: Universität Stuttgart. The sequence listing filed with the application follows.

SEQUENCE LISTING (36 sequences)

SEQ ID NO: 1 - protein, 111 aa, Homo sapiens
  SOURCE 1..111: /mol_type="protein" /organism="Homo sapiens"
AELPPKVSVFVPPRDGFFGNPRKSKLICQATGFSPRQIQVSWLREGKQVGSGVTTDQVQAEAKESGPTTYKVTSTLTIKESDWLGQSMFTCRVDHRGLTFQQNASSMCVPD

SEQ ID NO: 2 - protein, 106 aa, Homo sapiens
  SOURCE 1..106: /mol_type="protein" /organism="Homo sapiens"
DFTPPTVKILQSSCDGGGHFPPTIQLLCLVSGYTPGTINITWLEDGQVMDVDLSTASTTQEGELASTQSELTLSQKHWLSDRTYTCQVTYQGHTFEDSTKKCADSN

SEQ ID NO: 3 - protein, 265 aa, Homo sapiens
  SOURCE 1..265: /mol_type="protein" /organism="Homo sapiens"
MKYLLPTAAAGLLLLAAQPAMAEVQLVESGGGLVQPGGSLRLSCAASGFNIKDTYIHWVRQAPGKGLEWVARIYPTNGYTRYADSVKGRFTISADTSKNTAYLQMNSLRAEDTAVYYCSRWGGDGFYAMDYWGQGTLVTVSSGGGGSGGGGSGGGTGDIQMTQSPSSLSASVGDRVTITCRASQDVNTAVAWYQQKPGKAPKLLIYSASFLYSGVPSRFSGSRSGTDFTLTISSLQPEDFATYYCQQHYTTPPTFGQGTKVEIKR

SEQ ID NO: 4 - protein, 264 aa, Homo sapiens
  SOURCE 1..264: /mol_type="protein" /organism="Homo sapiens"
MKYLLPTAAAGLLLLAAQPAMAEVQLVESGGGLVQPGGSLRLSCAASGFSLTNYGVHWVRQAPGKGLEWLGVIWSGGNTDYNTPFTSRFTISRDNSKNTLYLQMNSLRAEDTAVYYCARALTYYDYEFAYWGQGTTVTVSSGGGGSGGGGSGGGGSDIQLTQSPSFLSASVGDRVTITCRASQSIGTNIHWYQQKPGKAPKLLIKYASESISGVPSRFSGSGSGTEFTLTISSLQPEDFATYYCQQNNNWPTTFGAGTKLEIKR

SEQ ID NO: 5 - protein, 472 aa, artificial sequences
  SOURCE 1..472: /mol_type="protein" /note="scTNF" /organism="artificial sequences"
SSRTPSDKPVAHVVANPQAEGQLQWLNRRANALLANGVELRDNQLVVPSEGLYLIYSQVLFKGQGCPSTHVLLTHTISRIAVSYQTKVNLLSAIKSPCQRETPEGAEAKPWYEPIYLGGVFQLEKGDRLSAEINRPDYLDFAESGQVYFGIIALGGGGSSSRTPSDKPVAHVVANPQAEGQLQWLNRRANALLANGVELRDNQLVVPSEGLYLIYSQVLFKGQGCPSTHVLLTHTISRIAVSYQTKVNLLSAIKSPCQRETPEGAEAKPWYEPIYLGGVFQLEKGDRLSAEINRPDYLDFAESGQVYFGIIALGGGGSSSRTPSDKPVAHVVANPQAEGQLQWLNRRANALLANGVELRDNQLVVPSEGLYLIYSQVLFKGQGCPSTHVLLTHTISRIAVSYQTKVNLLSAIKSPCQRETPEGAEAKPWYEPIYLGGVFQLEKGDRLSAEINRPDYLDFAESGQVYFGIIAL

SEQ ID NO: 6 - protein, 580 aa, artificial sequences
  SOURCE 1..580: /mol_type="protein" /note="scTRAIL" /organism="artificial sequences"
TRGTSEETISTVQEKQQNISPLVRERGPQRVAAHITGTRGRSNTLSSPNSKNEKALGRKINSWESSRSGHSFLSNLHLRNGELVIHEKGFYYIYSQTYFRFQEEIKENTKNDKQMVQYIYKYTSYPDPILLMKSARNSCWSKDAEYGLYSIYQGGIFELKENDRIFVSVTNEHLIDMDHEASFFGAFLVGGGGSGGGSTSEETISTVQEKQQNISPLVRERGPQRVAAHITGTRGRSNTLSSPNSKNEKALGRKINSWESSRSGHSFLSNLHLRNGELVIHEKGFYYIYSQTYFRFQEEIKENTKNDKQMVQYIYKYTSYPDPILLMKSARNSCWSKDAEYGLYSIYQGGIFELKENDRIFVSVTNEHLIDMDHEASFFGAFLVGGGGSGGGSTSEETISTVQEKQQNISPLVRERGPQRVAAHITGTRGRSNTLSSPNSKNEKALGRKINSWESSRSGHSFLSNLHLRNGELVIHEKGFYYIYSQTYFRFQEEIKENTKNDKQMVQYIYKYTSYPDPILLMKSARNSCWSKDAEYGLYSIYQGGIFELKENDRIFVSVTNEHLIDMDHEASFFGAFLVG

SEQ ID NO: 7 - protein, 410 aa, artificial sequences
  SOURCE 1..410: /mol_type="protein" /note="scFvEGFR-MHD2" /organism="artificial sequences"
METDTLLLWVLLLWVPGSTGDAAQPAMAEVQLVESGGGLVQPGGSLRLSCAASGFSLTNYGVHWVRQAPGKGLEWLGVIWSGGNTDYNTPFTSRFTISRDNSKNTLYLQMNSLRAEDTAVYYCARALTYYDYEFAYWGQGTTVTVSSGGGGSGGGGSGGGGSDIQLTQSPSFLSASVGDRVTITCRASQSIGTNIHWYQQKPGKAPKLLIKYASESISGVPSRFSGSGSGTEFTLTISSLQPEDFATYYCQQNNNWPTTFGAGTKLEIKRGSLGGSGGAELPPKVSVFVPPRDGFFGNPRKSKLICQATGFSPRQIQVSWLREGKQVGSGVTTDQVQAEAKESGPTTYKVTSTLTIKESDWLGQSMFTCRVDHRGLTFQQNASSMCVPDGGGSGGGTGSEFAAAHHHHHH

SEQ ID NO: 8 - protein, 413 aa, artificial sequences
  SOURCE 1..413: /mol_type="protein" /note="MHD2-scFvHER2" /organism="artificial sequences"
METDTLLLWVLLLWVPGSTGDAAQPASAGAGSLGGSGGAELPPKVSVFVPPRDGFFGNPRKSKLICQATGFSPRQIQVSWLREGKQVGSGVTTDQVQAEAKESGPTTYKVTSTLTIKESDWLGQSMFTCRVDHRGLTFQQNASSMCVPDGGGSGGGTGSGGEVQLVESGGGLVQPGGSLRLSCAASGFNIKDTYIHWVRQAPGKGLEWVARIYPTNGYTRYADSVKGRFTISADTSKNTAYLQMNSLRAEDTAVYYCSRWGGDGFYAMDYWGQGTLVTVSSGGGGSGGGGSGGGTGDIQMTQSPSSLSASVGDRVTITCRASQDVNTAVAWYQQKPGKAPKLLIYSASFLYSGVPSRFSGSRSGTDFTLTISSLQPEDFATYYCQQHYTTPPTFGQGTKVEIKRAAAHHHHHH

SEQ ID NO: 9 - protein, 653 aa, artificial sequences
  SOURCE 1..653: /mol_type="protein" /note="scFvEGFR-MHD2-scFvHER2" /organism="artificial sequences"
METDTLLLWVLLLWVPGSTGDAAQPAMAEVQLVESGGGLVQPGGSLRLSCAASGFSLTNYGVHWVRQAPGKGLEWLGVIWSGGNTDYNTPFTSRFTISRDNSKNTLYLQMNSLRAEDTAVYYCARALTYYDYEFAYWGQGTTVTVSSGGGGSGGGGSGGGGSDIQLTQSPSFLSASVGDRVTITCRASQSIGTNIHWYQQKPGKAPKLLIKYASESISGVPSRFSGSGSGTEFTLTISSLQPEDFATYYCQQNNNWPTTFGAGTKLEIKRGSLGGSGGAELPPKVSVFVPPRDGFFGNPRKSKLICQATGFSPRQIQVSWLREGKQVGSGVTTDQVQAEAKESGPTTYKVTSTLTIKESDWLGQSMFTCRVDHRGLTFQQNASSMCVPDGGGSGGGTGSGGEVQLVESGGGLVQPGGSLRLSCAASGFNIKDTYIHWVRQAPGKGLEWVARIYPTNGYTRYADSVKGRFTISADTSKNTAYLQMNSLRAEDTAVYYCSRWGGDGFYAMDYWGQGTLVTVSSGGGGSGGGGSGGGTGDIQMTQSPSSLSASVGDRVTITCRASQDVNTAVAWYQQKPGKAPKLLIYSASFLYSGVPSRFSGSRSGTDFTLTISSLQPEDFATYYCQQHYTTPPTFGQGTKVEIKRAAAHHHHHH

SEQ ID NO: 10 - protein, 648 aa, artificial sequences
  SOURCE 1..648: /mol_type="protein" /note="MHD2-scTNF" /organism="artificial sequences"
METDTLLLWVLLLWVPGSTGDAAQPASAGAGSLGGSGGAELPPKVSVFVPPRDGFFGNPRKSKLICQATGFSPRQIQVSWLREGKQVGSGVTTDQVQAEAKESGPTTYKVTSTLTIKESDWLGQSMFTCRVDHRGLTFQQNASSMCVPDGGGSGGGTGSEFMRGSHHHHHHGSASSSSRTPSDKPVAHVVANPQAEGQLQWLNRRANALLANGVELRDNQLVVPSEGLYLIYSQVLFKGQGCPSTHVLLTHTISRIAVSYQTKVNLLSAIKSPCQRETPEGAEAKPWYEPIYLGGVFQLEKGDRLSAEINRPDYLDFAESGQVYFGIIALGGGGSSSRTPSDKPVAHVVANPQAEGQLQWLNRRANALLANGVELRDNQLVVPSEGLYLIYSQVLFKGQGCPSTHVLLTHTISRIAVSYQTKVNLLSAIKSPCQRETPEGAEAKPWYEPIYLGGVFQLEKGDRLSAEINRPDYLDFAESGQVYFGIIALGGGGSSSRTPSDKPVAHVVANPQAEGQLQWLNRRANALLANGVELRDNQLVVPSEGLYLIYSQVLFKGQGCPSTHVLLTHTISRIAVSYQTKVNLLSAIKSPCQRETPEGAEAKPWYEPIYLGGVFQLEKGDRLSAEINRPDYLDFAESGQVYFGIIAL

SEQ ID NO: 11 - protein, 888 aa, artificial sequences
  SOURCE 1..888: /mol_type="protein" /note="scFvEGFR-MHD2-scTNF" /organism="artificial sequences"
METDTLLLWVLLLWVPGSTGDAAQPAMAEVQLVESGGGLVQPGGSLRLSCAASGFSLTNYGVHWVRQAPGKGLEWLGVIWSGGNTDYNTPFTSRFTISRDNSKNTLYLQMNSLRAEDTAVYYCARALTYYDYEFAYWGQGTTVTVSSGGGGSGGGGSGGGGSDIQLTQSPSFLSASVGDRVTITCRASQSIGTNIHWYQQKPGKAPKLLIKYASESISGVPSRFSGSGSGTEFTLTISSLQPEDFATYYCQQNNNWPTTFGAGTKLEIKRGSLGGSGGAELPPKVSVFVPPRDGFFGNPRKSKLICQATGFSPRQIQVSWLREGKQVGSGVTTDQVQAEAKESGPTTYKVTSTLTIKESDWLGQSMFTCRVDHRGLTFQQNASSMCVPDGGGSGGGTGSEFMRGSHHHHHHGSASSSSRTPSDKPVAHVVANPQAEGQLQWLNRRANALLANGVELRDNQLVVPSEGLYLIYSQVLFKGQGCPSTHVLLTHTISRIAVSYQTKVNLLSAIKSPCQRETPEGAEAKPWYEPIYLGGVFQLEKGDRLSAEINRPDYLDFAESGQVYFGIIALGGGGSSSRTPSDKPVAHVVANPQAEGQLQWLNRRANALLANGVELRDNQLVVPSEGLYLIYSQVLFKGQGCPSTHVLLTHTISRIAVSYQTKVNLLSAIKSPCQRETPEGAEAKPWYEPIYLGGVFQLEKGDRLSAEINRPDYLDFAESGQVYFGIIALGGGGSSSRTPSDKPVAHVVANPQAEGQLQWLNRRANALLANGVELRDNQLVVPSEGLYLIYSQVLFKGQGCPSTHVLLTHTISRIAVSYQTKVNLLSAIKSPCQRETPEGAEAKPWYEPIYLGGVFQLEKGDRLSAEINRPDYLDFAESGQVYFGIIAL

SEQ ID NO: 12 - protein, 724 aa, artificial sequences
  SOURCE 1..724: /mol_type="protein" /note="MHD2-scTRAIL" /organism="artificial sequences"
MDWTWRVFCLLAVAPGAHSLDDYKDDDDKEFAELPPKVSVFVPPRDGFFGNPRKSKLICQATGFSPRQIQVSWLREGKQVGSGVTTDQVQAEAKESGPTTYKVTSTLTIKESDWLGQSMFTCRVDHRGLTFQQNASSMCVPDEFTRGTSEETISTVQEKQQNISPLVRERGPQRVAAHITGTRGRSNTLSSPNSKNEKALGRKINSWESSRSGHSFLSNLHLRNGELVIHEKGFYYIYSQTYFRFQEEIKENTKNDKQMVQYIYKYTSYPDPILLMKSARNSCWSKDAEYGLYSIYQGGIFELKENDRIFVSVTNEHLIDMDHEASFFGAFLVGGGGSGGGSTSEETISTVQEKQQNISPLVRERGPQRVAAHITGTRGRSNTLSSPNSKNEKALGRKINSWESSRSGHSFLSNLHLRNGELVIHEKGFYYIYSQTYFRFQEEIKENTKNDKQMVQYIYKYTSYPDPILLMKSARNSCWSKDAEYGLYSIYQGGIFELKENDRIFVSVTNEHLIDMDHEASFFGAFLVGGGGSGGGSTSEETISTVQEKQQNISPLVRERGPQRVAAHITGTRGRSNTLSSPNSKNEKALGRKINSWESSRSGHSFLSNLHLRNGELVIHEKGFYYIYSQTYFRFQEEIKENTKNDKQMVQYIYKYTSYPDPILLMKSARNSCWSKDAEYGLYSIYQGGIFELKENDRIFVSVTNEHLIDMDHEASFFGAFLVG

SEQ ID NO: 13 - protein, 978 aa, artificial sequences
  SOURCE 1..978: /mol_type="protein" /note="scFvEGFR-MHD2-scTRAIL" /organism="artificial sequences"
METDTLLLWVLLLWVPGSTGDYKDDDDKGGGGSAAQPAMAEVQLVESGGGLVQPGGSLRLSCAASGFSLTNYGVHWVRQAPGKGLEWLGVIWSGGNTDYNTPFTSRFTISRDNSKNTLYLQMNSLRAEDTAVYYCARALTYYDYEFAYWGQGTTVTVSSGGGGSGGGGSGGGGSDIQLTQSPSFLSASVGDRVTITCRASQSIGTNIHWYQQKPGKAPKLLIKYASESISGVPSRFSGSGSGTEFTLTISSLQPEDFATYYCQQNNNWPTTFGAGTKLEIKRAAAAELPPKVSVFVPPRDGFFGNPRKSKLICQATGFSPRQIQVSWLREGKQVGSGVTTDQVQAEAKESGPTTYKVTSTLTIKESDWLGQSMFTCRVDHRGLTFQQNASSMCVPDEFTRGTSEETISTVQEKQQNISPLVRERGPQRVAAHITGTRGRSNTLSSPNSKNEKALGRKINSWESSRSGHSFLSNLHLRNGELVIHEKGFYYIYSQTYFRFQEEIKENTKNDKQMVQYIYKYTSYPDPILLMKSARNSCWSKDAEYGLYSIYQGGIFELKENDRIFVSVTNEHLIDMDHEASFFGAFLVGGGGSGGGSTSEETISTVQEKQQNISPLVRERGPQRVAAHITGTRGRSNTLSSPNSKNEKALGRKINSWESSRSGHSFLSNLHLRNGELVIHEKGFYYIYSQTYFRFQEEIKENTKNDKQMVQYIYKYTSYPDPILLMKSARNSCWSKDAEYGLYSIYQGGIFELKENDRIFVSVTNEHLIDMDHEASFFGAFLVGGGGSGGGSTSEETISTVQEKQQNISPLVRERGPQRVAAHITGTRGRSNTLSSPNSKNEKALGRKINSWESSRSGHSFLSNLHLRNGELVIHEKGFYYIYSQTYFRFQEEIKENTKNDKQMVQYIYKYTSYPDPILLMKSARNSCWSKDAEYGLYSIYQGGIFELKENDRIFVSVTNEHLIDMDHEASFFGAFLVG

SEQ ID NO: 14 - protein, 1217 aa, artificial sequences [sequence omitted]

SEQ ID NO: 15 - protein, 405 aa, artificial sequences
  SOURCE 1..405: /mol_type="protein" /note="scFvEGFR-EHD2" /organism="artificial sequences"
METDTLLLWVLLLWVPGSTGDAAQPAMAEVQLVESGGGLVQPGGSLRLSCAASGFSLTNYGVHWVRQAPGKGLEWLGVIWSGGNTDYNTPFTSRFTISRDNSKNTLYLQMNSLRAEDTAVYYCARALTYYDYEFAYWGQGTTVTVSSGGGGSGGGGSGGGGSDIQLTQSPSFLSASVGDRVTITCRASQSIGTNIHWYQQKPGKAPKLLIKYASESISGVPSRFSGSGSGTEFTLTISSLQPEDFATYYCQQNNNWPTTFGAGTKLEIKRGSLGGSGGDFTPPTVKILQSSCDGGGHFPPTIQLLCLVSGYTPGTINITWLEDGQVMDVDLSTASTTQEGELASTQSELTLSQKHWLSDRTYTCQVTYQGHTFEDSTKKCADSNGGGSGGGTGSEFAAAHHHHHH

SEQ ID NO: 16 - protein, 731 aa, artificial sequences
  SOURCE 1..731: /mol_type="protein" /note="EHD2-scTRAIL" /organism="artificial sequences"
METDTLLLWVLLLWVPGSTGDYKDDDDKGGGGSAAQPADFTPPTVKILQSSCDGGGHFPPTIQLLCLVSGYTPGTINITWLEDGQVMDVDLSTASTTQEGELASTQSELTLSQKHWLSDRTYTCQVTYQGHTFEDSTKKCADSNGGSGGEFTRGTSEETISTVQEKQQNISPLVRERGPQRVAAHITGTRGRSNTLSSPNSKNEKALGRKINSWESSRSGHSFLSNLHLRNGELVIHEKGFYYIYSQTYFRFQEEIKENTKNDKQMVQYIYKYTSYPDPILLMKSARNSCWSKDAEYGLYSIYQGGIFELKENDRIFVSVTNEHLIDMDHEASFFGAFLVGGGGSGGGSTSEETISTVQEKQQNISPLVRERGPQRVAAHITGTRGRSNTLSSPNSKNEKALGRKINSWESSRSGHSFLSNLHLRNGELVIHEKGFYYIYSQTYFRFQEEIKENTKNDKQMVQYIYKYTSYPDPILLMKSARNSCWSKDAEYGLYSIYQGGIFELKENDRIFVSVTNEHLIDMDHEASFFGAFLVGGGGSGGGSTSEETISTVQEKQQNISPLVRERGPQRVAAHITGTRGRSNTLSSPNSKNEKALGRKINSWESSRSGHSFLSNLHLRNGELVIHEKGFYYIYSQTYFRFQEEIKENTKNDKQMVQYIYKYTSYPDPILLMKSARNSCWSKDAEYGLYSIYQGGIFELKENDRIFVSVTNEHLIDMDHEASFFGAFLVG

SEQ ID NO: 17 - protein, 983 aa, artificial sequences [sequence omitted]

SEQ ID NO: 18 - protein, 5 aa, artificial sequences
  SOURCE 1..5: /mol_type="protein" /note="peptide linker 1" /organism="artificial sequences"
GGGGS

SEQ ID NO: 19 - protein, 10 aa, artificial sequences
  SOURCE 1..10: /mol_type="protein" /note="peptide linker 2" /organism="artificial sequences"
GGGGSGGGGS

SEQ ID NO: 20 - protein, 15 aa, artificial sequences
  SOURCE 1..15: /mol_type="protein" /note="peptide linker 3" /organism="artificial sequences"
GGGGSGGGGSGGGGS

SEQ ID NO: 21 - protein, 8 aa, artificial sequences
  SOURCE 1..8: /mol_type="protein" /note="peptide linker 4" /organism="artificial sequences"
GSLGGSGG

SEQ ID NO: 22 - protein, 8 aa, artificial sequences
  SOURCE 1..8: /mol_type="protein" /note="peptide linker 5" /organism="artificial sequences"
GGGSGGGT

SEQ ID NO: 23 - protein, 10 aa, artificial sequences
  SOURCE 1..10: /mol_type="protein" /note="peptide linker 6" /organism="artificial sequences"
GGGSGGGTGS

SEQ ID NO: 24 - protein, 12 aa, artificial sequences
  SOURCE 1..12: /mol_type="protein" /note="peptide linker 7" /organism="artificial sequences"
GGGSGGGTGSGG

SEQ ID NO: 25 - protein, 8 aa, artificial sequences
  SOURCE 1..8: /mol_type="protein" /note="peptide linker 8" /organism="artificial sequences"
GGGSGGGS

SEQ ID NO: 26 - protein, 5 aa, artificial sequences
  SOURCE 1..5: /mol_type="protein" /note="peptide linker 9" /organism="artificial sequences"
EFTRG

SEQ ID NO: 27 - protein, 3 aa, artificial sequences
  SOURCE 1..3: /mol_type="protein" /note="peptide linker 10" /organism="artificial sequences"
AAA

SEQ ID NO: 28 - protein, 405 aa, artificial sequences
  SOURCE 1..405: /mol_type="protein" /note="Anti-CEA scFv-EHD2" /organism="artificial sequences"
METDTLLLWVLLLWVPGSTGDAAQPAMAQVKLQQSGAELVRSGTSVKLSCTASGFNIKDSYMHWLRQGPEQGLEWIGWIDPENGDTEYAPKFQGKATFTTDTSSNTAYLQLSSLTSEDTAVYYCNEGTPTGPYYFDYWGQGTTVTVSSGGGGSGGGGSGGGGSDIELTQSPAIMSASPGEKVTITCSASSSVSYMHWFQQKPGTSPKLWIYSTSNLASGVPARFSGSGSGTSYSLTISRMEAEDAATYYCQQRSSYPLTFGAGTKLELKRGSLGGSGGDFTPPTVKILQSSCDGGGHFPPTIQLLCLVSGYTPGTINITWLEDGQVMDVDLSTASTTQEGELASTQSELTLSQKHWLSDRTYTCQVTYQGHTFEDSTKKCADSNGGGSGGGTGSEFAAAHHHHHH

SEQ ID NO: 29 - protein, 391 aa, artificial sequences
  SOURCE 1..391: /mol_type="protein" /note="Anti-HER2 scFv-EHD2" /organism="artificial sequences"
METDTLLLWVLLLWVPGSTGEVQLVESGGGLVQPGGSLRLSCAASGFNIKDTYIHWVRQAPGKGLEWVARIYPTNGYTRYADSVKGRFTISADTSKNTAYLQMNSLRAEDTAVYYCSRWGGDGFYAMDYWGQGTLVTVSSGGGGSGGGGSGGGGSDIQMTQSPSSLSASVGDRVTITCRASQDVNTAVAWYQQKPGKAPKLLIYSASFLYSGVPSRFSGSRSGTDFTLTISSLQPEDFATYYCQQHYTTPPTFGQGTKVEIKRAAAGGSGGDFTPPTVKILQSSCDGGGHFPPTIQLLCLVSGYTPGTINITWLEDGQVMDVDLSTASTTQEGELASTQSELTLSQKHWLSDRTYTCQVTYQGHTFEDSTKKCADSNGGSGGASSHHHHHH

SEQ ID NO: 30 - protein, 393 aa, artificial sequences
  SOURCE 1..393: /mol_type="protein" /note="Anti-HER3 scFv-EHD2" /organism="artificial sequences"
METDTLLLWVLLLWVPGSTGEVQLLESGGGLVQPGGSLRLSCAASGFTFSHYVMAWVRQAPGKGLEWVSSISSSGGWTLYADSVKGRFTISRDNSKNTLYLQMNSLRAEDTAVYYCTRGLKMATIFDYWGQGTLVTVSSGGGGSGGGGSGGGGSQSALTQPASVSGSPGQSITISCTGTSSDVGSYNVVSWYQQHPGKAPKLIIYEVSQRPSGVSNRFSGSKSGNTASLTISGLQTEDEADYYCSSYAGSSIFVIFGGGTKVTVLAAAGGSGGDFTPPTVKILQSSCDGGGHFPPTIQLLCLVSGYTPGTINITWLEDGQVMDVDLSTASTTQEGELASTQSELTLSQKHWLSDRTYTCQVTYQGHTFEDSTKKCADSNGGSGGASSHHHHHH

SEQ ID NO: 31 - protein, 645 aa, artificial sequences
  SOURCE 1..645: /mol_type="protein" /note="Anti-CEAxCD3 scDb-EHD2" /organism="artificial sequences"
METDTLLLWVLLLWVPGSTGDAAQPAMAQVKLQQSGAELVRSGTSVKLSCTASGFNIKDSYMHWLRQGPEQGLEWIGWIDPENGDTEYAPKFQGKATFTTDTSSNTAYLQLSSLTSEDTAVYYCNEGTPTGPYYFDYWGQGTTVTVSSGGGGSDIQMTQSPSSLSASVGDRVTITCRASQDIRNYLNWYQQKPGKAPKLLIYYTSRLESGVPSRFSGSGSGTDYTLTISSLQPEDFATYYCQQGNTLPWTFGQGTKVEIKRGGGGSGGRASGGGGSEVQLVESGGGLVQPGGSLRLSCAASGYSFTGYTMNWVRQAPGKGLEWVALINPYKGVSTYNQKFKDRFTISVDKSKNTAYLQMNSLRAEDTAVYYCARSGYYGDSDWYFDVWGQGTLVTVSSGGGGSDIELTQSPAIMSASPGEKVTITCSASSSVSYMHWFQQKPGTSPKLWIYSTSNLASGVPARFSGSGSGTSYSLTISRMEAEDAATYYCQQRSSYPLTFGAGTKLELKRGSLGGSGGDFTPPTVKILQSSCDGGGHFPPTIQLLCLVSGYTPGTINITWLEDGQVMDVDLSTASTTQEGELASTQSELTLSQKHWLSDRTYTCQVTYQGHTFEDSTKKCADSNGGGSGGGTGSEFAAAHHHHHH

SEQ ID NO: 32 - protein, 394 aa, artificial sequences
  SOURCE 1..394: /mol_type="protein" /note="Anti-EGFR scFv-L3-EHD2" /organism="artificial sequences"
METDTLLLWVLLLWVPGSTGQVQLKQSGAELVKPGASVKLSCKTSGYTFTENIIHWVKQRSGQGLEWIGWFHPGSGSIKYNEKFKDKATLTADKSSSTVYMELSRLTSEDSAVYFCARHGGTGRGAMDYWGQGTSVTVSSGGCGSGGGGSGGSAQILMTQSPASSVVSLGQRATISCRASKSVSTSAYSYMHWYQQKPGQPPKLLIYLASNLESGVPPRFSGSGSGTDFTLNIHPVEEEDAATYYCQHSRELPYTFGGGTKLEIKRAAAGGSGGDFTPPTVKILQSSCDGGGHFPPTIQLLCLVSGYTPGTINITWLEDGQVMDVDLSTASTTQEGELASTQSELTLSQKHWLSDRTYTCQVTYQGHTFEDSTKKCADSNGGSGGASSHHHHHH

SEQ ID NO: 33 - protein, 645 aa, artificial sequences
  SOURCE 1..645: /mol_type="protein" /note="Anti-EGFR scFv-L3-EHD2-scFv" /organism="artificial sequences"
METDTLLLWVLLLWVPGSTGQVQLKQSGAELVKPGASVKLSCKTSGYTFTENIIHWVKQRSGQGLEWIGWFHPGSGSIKYNEKFKDKATLTADKSSSTVYMELSRLTSEDSAVYFCARHGGTGRGAMDYWGQGTSVTVSSGGCGSGGGGSGGSAQILMTQSPASSVVSLGQRATISCRASKSVSTSAYSYMHWYQQKPGQPPKLLIYLASNLESGVPPRFSGSGSGTDFTLNIHPVEEEDAATYYCQHSRELPYTFGGGTKLEIKRAAAGGSGGDFTPPTVKILQSSCDGGGHFPPTIQLLCLVSGYTPGTINITWLEDGQVMDVDLSTASTTQEGELASTQSELTLSQKHWLSDRTYTCQVTYQGHTFEDSTKKCADSNGGSGGASSEFQVQLKQSGAELVKPGASVKLSCKTSGYTFTENIIHWVKQRSGQGLEWIGWFHPGSGSIKYNEKFKDKATLTADKSSSTVYMELSRLTSEDSAVYFCARHGGTGRGAMDYWGQGTSVTVSSGGGGSGGGGSGGSAQILMTQSPASSVVSLGQRATISCRASKSVSTSAYSYMHWYQQKPGQPPKLLIYLASNLESGVPPRFSGSGSGTDFTLNIHPVEEEDAATYYCQHSRELPYTFGGGTKLEIKRAAAHHHHHH

SEQ ID NO: 34 - protein, 652 aa, artificial sequences
  SOURCE 1..652: /mol_type="protein" /note="MHD2-scTNFR2" /organism="artificial sequences"
METDTLLLWVLLLWVPGSTGDAAQPAGGGAAAHHHHHHGGTGGGGSGGKLGGSGGAELPPKVSVFVPPRDGFFGNPRKSKLICQATGFSPRQIQVSWLREGKQVGSGVTTDQVQAEAKESGPTTYKVTSTLTIKESDWLGQSMFTCRVDHRGLTFQQNASSMCVPDGGGSGGGTGSEFLASSRTPSDKPVAHVVANPQAEGQLQWLNRRANALLANGVELRDNQLVVPSEGLYLIYSQVLFKGQGCPSTHVLLTHTISRIAVSYQTKVNLLSAIKSPCQRETPEGAEAKPWYEPIYLGGVFQLEKGDRLSAEINRPDYLNFRESGQVYFGIIALGGGGSSSRTPSDKPVAHVVANPQAEGQLQWLNRRANALLANGVELRDNQLVVPSEGLYLIYSQVLFKGQGCPSTHVLLTHTISRIAVSYQTKVNLLSAIKSPCQRETPEGAEAKPWYEPIYLGGVFQLEKGDRLSAEINRPDYLNFRESGQVYFGIIALGGGGSSSRTPSDKPVAHVVANPQAEGQLQWLNRRANALLANGVELRDNQLVVPSEGLYLIYSQVLFKGQGCPSTHVLLTHTISRIAVSYQTKVNLLSAIKSPCQRETPEGAEAKPWYEPIYLGGVFQLEKGDRLSAEINRPDYLNFRESGQVYFGIIAL

SEQ ID NO: 35 - protein, 647 aa, artificial sequences
  SOURCE 1..647: /mol_type="protein" /note="EHD2-scTNFR2-L16aa" /organism="artificial sequences"
METDTLLLWVLLLWVPGSTGDAAQPAGGGAAAHHHHHHGGTGGGGSGGKLGGSGGDFTPPTVKILQSSCDGGGHFPPTIQLLCLVSGYTPGTINITWLEDGQVMDVDLSTASTTQEGELASTQSELTLSQKHWLSDRTYTCQVTYQGHTFEDSTKKCADSNGGGSGGGTGSEFLASSRTPSDKPVAHVVANPQAEGQLQWLNRRANALLANGVELRDNQLVVPSEGLYLIYSQVLFKGQGCPSTHVLLTHTISRIAVSYQTKVNLLSAIKSPCQRETPEGAEAKPWYEPIYLGGVFQLEKGDRLSAEINRPDYLNFRESGQVYFGIIALGGGGSSSRTPSDKPVAHVVANPQAEGQLQWLNRRANALLANGVELRDNQLVVPSEGLYLIYSQVLFKGQGCPSTHVLLTHTISRIAVSYQTKVNLLSAIKSPCQRETPEGAEAKPWYEPIYLGGVFQLEKGDRLSAEINRPDYLNFRESGQVYFGIIALGGGGSSSRTPSDKPVAHVVANPQAEGQLQWLNRRANALLANGVELRDNQLVVPSEGLYLIYSQVLFKGQGCPSTHVLLTHTISRIAVSYQTKVNLLSAIKSPCQRETPEGAEAKPWYEPIYLGGVFQLEKGDRLSAEINRPDYLNFRESGQVYFGIIAL

SEQ ID NO: 36 - protein, 660 aa, artificial sequences
  SOURCE 1..660: /mol_type="protein" /note="EHD2-scTNFR2-L28aa" /organism="artificial sequences"
METDTLLLWVLLLWVPGSTGDAAQPAGGGAAAHHHHHHGGTGGGGSGGKLGGSGGDFTPPTVKILQSSCDGGGHFPPTIQLLCLVSGYTPGTINITWLEDGQVMDVDLSTASTTQEGELASTQSELTLSQKHWLSDRTYTCQVTYQGHTFEDSTKKCADSNGGGSGGGSGGGSGGGSGGGSGGSEFLASSRTPSDKPVAHVVANPQAEGQLQWLNRRANALLANGVELRDNQLVVPSEGLYLIYSQVLFKGQGCPSTHVLLTHTISRIAVSYQTKVNLLSAIKSPCQRETPEGAEAKPWYEPIYLGGVFQLEKGDRLSAEINRPDYLNFRESGQVYFGIIALGGGGSSSRTPSDKPVAHVVANPQAEGQLQWLNRRANALLANGVELRDNQLVVPSEGLYLIYSQVLFKGQGCPSTHVLLTHTISRIAVSYQTKVNLLSAIKSPCQRETPEGAEAKPWYEPIYLGGVFQLEKGDRLSAEINRPDYLNFRESGQVYFGIIALGGGGSSSRTPSDKPVAHVVANPQAEGQLQWLNRRANALLANGVELRDNQLVVPSEGLYLIYSQVLFKGQGCPSTHVLLTHTISRIAVSYQTKVNLLSAIKSPCQRETPEGAEAKPWYEPIYLGGVFQLEKGDRLSAEINRPDYLNFRESGQVYFGIIAL